European Patent Application EP 4 725 954 A1, published April 15, 2026. Title: 具有抗衰老和修复作用的多肽LA-19和TM-19等改构肽及其用途. Applicant: 安徽德馨华海生物科技有限公司. Application WO. The sequence listing filed with the application follows.

SEQUENCE LISTING (10 sequences)

SEQ ID NO: 1 - protein, 19 aa, synthetic construct
LQSSLRALRQMGGGTKAAA

SEQ ID NO: 2 - protein, 19 aa, synthetic construct
TKAAAGGGLQSSLRALRQM

SEQ ID NO: 3 - protein, 14 aa, synthetic construct
LQSSLRALRQMGGG

SEQ ID NO: 4 - protein, 14 aa, synthetic construct
GGGLQSSLRALRQM

SEQ ID NO: 5 - protein, 11 aa, synthetic construct
LQSSLRALRQM

SEQ ID NO: 6 - protein, 19 aa, synthetic construct
LQSSLRALRQMGGGTKAAA

SEQ ID NO: 7 - protein, 19 aa, synthetic construct
LQSSLRALRQMGGGTKAAA

SEQ ID NO: 8 - protein, 19 aa, synthetic construct
LQTSLRALRQIGGGTKAAA

SEQ ID NO: 9 - protein, 19 aa, synthetic construct
LQTSLRALRQIGGGTKAAA

SEQ ID NO: 10 - protein, 19 aa, synthetic construct
TKAAAGGGLQTSLRALRQI